European Patent Application EP 4 726 041 A1, published April 15, 2026. Title: MED12 INHIBITOR, OR PHARMACEUTICAL COMPOSITION COMPRISING THEREOF, FOR USE IN A METHOD FOR THE TREATMENT OF CANCER. Applicant: INSTITUTO DE INVESTIGACIÓN BIOMÉDICA DE SALAMANCA DE LA FUNDACIÓN INSTITUTO CIENCIAS DE LA SALUD DE CASTILLA Y LEÓN. The sequence listing filed with the application follows.

SEQUENCE LISTING (15 sequences)

SEQ ID NO: 1 - RNA, 20 nt, synthetic construct
  source 1..20: mol_type = other RNA
acggccttgaatgtaaaaca

SEQ ID NO: 2 - RNA, 20 nt, synthetic construct
  source 1..20: mol_type = other RNA
ataaccagcctgctgtctct

SEQ ID NO: 3 - RNA, 25 nt, synthetic construct
  source 1..25: mol_type = other RNA
caccgacggccttgaatgtaaaaca

SEQ ID NO: 4 - RNA, 25 nt, synthetic construct
  source 1..25: mol_type = other RNA
caccgataaccagcctgctgtctct

SEQ ID NO: 5 - RNA, 26 nt, synthetic construct
  source 1..26: mol_type = other RNA
aaactgttttacacttcaaggccgtc

SEQ ID NO: 6 - RNA, 25 nt, synthetic construct
  source 1..25: mol_type = other RNA
aaacagagacagcaggcyggttatc

SEQ ID NO: 7 - RNA, 21 nt, synthetic construct
  source 1..21: mol_type = other RNA
ggttaagaagagacatgttga

SEQ ID NO: 8 - RNA, 21 nt, synthetic construct
  source 1..21: mol_type = other RNA
gctggccatgttcatgtttca

SEQ ID NO: 9 - RNA, 21 nt, synthetic construct
  source 1..21: mol_type = other RNA
gctgttctgtgaactgattcg

SEQ ID NO: 10 - DNA, 21 bp, synthetic construct
  source 1..21: mol_type = other DNA
tcctagtgaccatgggagtga

SEQ ID NO: 11 - DNA, 21 bp, synthetic construct
  source 1..21: mol_type = other DNA
ggtcatgaaggcaaactcagc

SEQ ID NO: 12 - DNA, 21 bp, synthetic construct
  source 1..21: mol_type = other DNA
cgggatcttgagctacgaaca

SEQ ID NO: 13 - DNA, 20 bp, synthetic construct
  source 1..20: mol_type = other DNA
tccttctggttcacttgggg

SEQ ID NO: 14 - DNA, 20 bp, synthetic construct
  source 1..20: mol_type = other DNA
agccagccttcactggagat

SEQ ID NO: 15 - DNA, 20 bp, synthetic construct
  source 1..20: mol_type = other DNA
ctgggatcgagcagtaacca